European Patent Application EP 4 116 426 A1, published January 11, 2023. Title: Method and System for Multiplex Genome Editing. Applicant: Suzhou Qi Biodesign Biotechnology Company Limited. Application EP EP 21764356.8. The sequence listing filed with the application follows.

SEQUENCE LISTING (48 sequences)

SEQ ID NO: 1 - protein, 438 aa, artificial sequence
AGTAATTCATCCAGGTCACCAAGTTCTAGGATTTTCAGAACTGCAACTTATTTTATCAAGGAATCTTTAAACATACGAACAGATCACTTAAAGTTCTTCTGAAGCAACTTAAAGTTATCAGGCATGCATGGATCTTGGAGGAATCAGATGTGCAGTCAGGGACCATAGCACAAGACAGGCGTCTTCTACTGGTGCTACCAGCAAATGCTGGAAGCCGGGAACACTGGGTACGTTGGAAACCACGTGATGTGAAGAAGTAAGATAAACTGTAGGAGAAAAGCATTTCGTAGTGGGCCATGAAGCCTTTCAGGACATGTATTGCAGTATGGGCCGGCCCATTACGCAATTGGACGACAACAAAGACTAGTATTAGTACCACCTCGGCTATCCACATAGATCAAAGCTGATTTAAAAGAGTTGTGCAGATGATCCGTGGCG

SEQ ID NO: 2 - protein, 361 aa, artificial sequence
GACCAAGCCCGTTATTCTGACAGTTCTGGTGCTCAACACATTTATATTTATCAAGGAGCACATTGTTACTCACTGCTAGGAGGGAATCGAACTAGGAATATTGATCAGAGGAACTACGAGAGAGCTGAAGATAACTGCCCTCTAGCTCTCACTGATCTGGGCGCATAGTGAGATGCAGCCCACGTGAGTTCAGCAACGGTCTAGCGCTGGGCTTTTAGGCCCGCATGATCGGGCTTTGTCGGGTGGTCGACGTGTTCACGATTGGGGAGAGCAACGCAGCAGTTCCTCTTAGTTTAGTCCCACCTCGCCTGTCCAGCAGAGTTCTGACCGGTTTATAAACTCGCTTGCTGCATCAGACTTG

SEQ ID NO: 3 - protein, 96 aa, artificial sequence
GTTTTAGAGCTAGAAATAGCAAGTTAAAATAAGGCTAGTCCGTTATCAACTTGAAAAAGTGGCACCGAGTCGGTGCTTTTTTTGTTTTTTATGTCT

SEQ ID NO: 4 - protein, 106 aa, artificial sequence
GTTTAAGAGCTATGCTGGAAACAGCATAGCAAGTTTAAATAAGGCTAGTCCGTTATCAACTTGAAAAAGTGGCACCGAGTCGGTGCTTTTTTTGTTTTTTATGTCT

SEQ ID NO: 5 - protein, 156 aa, artificial sequence
GTTTTAGAGCTAGGCCAACATGAGGATCACCCATGTCTGCAGGGCCTAGCAAGTTAAAATAAGGCTAGTCCGTTATCAACTTGGCCAACATGAGGATCACCCATGTCTGCAGGGCCAAGTGGCACCGAGTCGGTGCTTTTTTTGTTTTTTATGTCT

SEQ ID NO: 6 - protein, 156 aa, artificial sequence
GTTTAAGAGCTAGGCCAAGATGAGGATCACCCATGCCTGCAGGGCCTAGCAAGTTTAAATAAGGCTAGTCCGTTATCAACTTGGCCAACATGAGGATCACCCATGTCTGCAGGGCCAAGTGGCACCGAGTCGGTGCTTTTTTTGTTTTTTATGTCT

SEQ ID NO: 7 - protein, 156 aa, artificial sequence
GTTTCAGAGCTAGGCCAAGATGAGGATCACCCATGCCTGCAGGGCCTAGCAAGTTGAAATAAGGCTAGTCCGTTATCAACTTGGCCAACATGAGGATCACCCATGTCTGCAGGGCCAAGTGGCACCGAGTCGGTGCTTTTTTTGTTTTTTATGTCT

SEQ ID NO: 8 - protein, 158 aa, artificial sequence
GTTTAAGAGCTATGCTGAAGATGAGGATCACCCATGCCTGCAGCAGCATAGCAAGTTTAAATAAGGCTAGTCCGTTATCAACTTGGCCAACATGAGGATCACCCATGTCTGCAGGGCCAAGTGGCACCGAGTCGGTGCTTTTTTTGTTTTTTATGTCT

SEQ ID NO: 9 - protein, 158 aa, artificial sequence
GTTTCAGAGCTATGCTGAAGATGAGGATCACCCATGCCTGCAGCAGCATAGCAAGTTGAAATAAGGCTAGTCCGTTATCAACTTGGCCAACATGAGGATCACCCATGTCTGCAGGGCCAAGTGGCACCGAGTCGGTGCTTTTTTTGTTTTTTATGTCT

SEQ ID NO: 10 - protein, 223 aa, artificial sequence
GTTTTAGAGCTAGGCCAACATGAGGATCACCCATGTCTGCAGGGCCTAGCAAGTTAAAATAAGGCTAGTCCGTTATCAACTTGGCCAACATGAGGATCACCCATGTCTGCAGGGCCAAGTGGCACCGAGTCGGTGCGGGAGCACATGAGGATCACCCATGTGCCACGAGCGACATGAGGATCACCCATGTCGCTCGTGTTCCCTTTTTTTGTTTTTTATGTCT

SEQ ID NO: 11 - protein, 163 aa, artificial sequence
GTTTTAGAGCTAGAAATAGCAAGTTAAAATAAGGCTAGTCCGTTATCAACTTGAAAAAGTGGCACCGAGTCGGTGCGGGAGCACATGAGGATCACCCATGTGCCACGAGCGACATGAGGATCACCCATGTCGCTCGTGTTCCCTTTTTTTGTTTTTTATGTCT

SEQ ID NO: 12 - protein, 131 aa, artificial sequence
GTTTAAGAGCTATGCTGGAAACAGCATAGCAAGTTTAAATAAGGCTAGTCCGTTATCAACTTGAAAAAGTGGCACCGAGTCGGTGCGCGCACATGAGGATCACCCATGTGCTTTTTTTGTTTTTTATGTCT

SEQ ID NO: 13 - protein, 173 aa, artificial sequence
GTTTAAGAGCTATGCTGGAAACAGCATAGCAAGTTTAAATAAGGCTAGTCCGTTATCAACTTGAAAAAGTGGCACCGAGTCGGTGCGGGAGCACATGAGGATCACCCATGTGCCACGAGCGACATGAGGATCACCCATGTCGCTCGTGTTCCCTTTTTTTGTTTTTTATGTCT

SEQ ID NO: 14 - protein, 162 aa, artificial sequence
GTTTAAGAGCTATGCTGGAAACAGCATAGCAAGTTTAAATAAGGCTAGTCCGTTATCAACTTGAAAAAGTGGCACCGAGTCGGTGCGGGAGCACATGAGGATCACCCATGTGCGACTCCCACAGTCACTGGGGAGTCTTCCCTTTTTTTGTTTTTTATGTCT

SEQ ID NO: 15 - protein, 216 aa, artificial sequence
GTTTAAGAGCTATGCTGGAAACAGCATAGCAAGTTTAAATAAGGCTAGTCCGTTATCAACTTGAAAAAGTGGCACCGAGTCGGTGCGGGAGCACATGAGGATCACCCATGTGCCACGAGCGACATGAGGATCACCCATGTCGCTCGTGGACTCTCGTGTCACATGAGGATCACCCATGTGACACGAGAGTCTTCCCTTTTTTTGTTTTTTATGTCT

SEQ ID NO: 16 - protein, 142 aa, artificial sequence
GTTTGAGAGCTACCTAAGGAGTTTATATGGAAACCCTTAGGTAGCAAGTTCAAATAAGGCTAGTCCGTTATCAACTTTAAGGAGTTTATATGGAAACCCTTAAAGTGGCACCGAGTCGGTGCTTTTTTTGTTTTTTATGTCT

SEQ ID NO: 17 - protein, 142 aa, artificial sequence
GTTTGAGAGCTACCGGAGCAGACGATATGGCGTCGCTCCGGTAGCAAGTTCAAATAAGGCTAGTCCGTTATCAACTTGGAGCAGACGATATGGCGTCGCTCCAAGTGGCACCGAGTCGGTGCTTTTTTTGTTTTTTATGTCT

SEQ ID NO: 18 - protein, 137 aa, artificial sequence
GTTTAAGAGCTATGCTGGAAACAGCATAGCAAGTTTAAATAAGGCTAGTCCGTTATCAACTTGAAAAAGTGGCACCGAGTCGGTGCAACATAAGGAGTTTATATGGAAACCCTTATGTTTTTTTGTTTTTTATGTCT

SEQ ID NO: 19 - protein, 185 aa, artificial sequence
GTTTAAGAGCTATGCTGGAAACAGCATAGCAAGTTTAAATAAGGCTAGTCCGTTATCAACTTGAAAAAGTGGCACCGAGTCGGTGCGGGAGCTAAGGAGTTTATATGGAAACCCTTAGCCTGCTGCGTAAGGAGTTTATATGGAAACCCTTACGCAGCAGTTCCCTTTTTTTGTTTTTTATGTCT

SEQ ID NO: 20 - protein, 185 aa, artificial sequence
GTTTAAGAGCTATGCTGGAAACAGCATAGCAAGTTTAAATAAGGCTAGTCCGTTATCAACTTGAAAAAGTGGCACCGAGTCGGTGCGGGAGCGGAGCAGACGATATGGCGTCGCTCCGCCTGCTGCGGGAGCAGACGATATGGCGTCGCTCCCGCAGCAGTTCCCTTTTTTTGTTTTTTATGTCT

SEQ ID NO: 21 - protein, 126 aa, artificial sequence
GTTTGAGAGCTAGGGCCCTGAAGAAGGGCCCTAGCAAGTTCAAATAAGGCTAGTCCGTTATCAACTTGGGCCCTGAAGAAGGGCCCAAGTGGCACCGAGTCGGTGCTTTTTTTGTTTTTTATGTCT

SEQ ID NO: 22 - protein, 165 aa, artificial sequence
GTTTAAGAGCTATGCTGGAAACAGCATAGCAAGTTTAAATAAGGCTAGTCCGTTATCAACTTGAAAAAGTGGCACCGAGTCGGTGCGGGAGCGCCCTGAAGAAGGGCGCCTGCTGCGGCCCTGAAGAAGGGCCGCAGCAGTTCCCTTTTTTTGTTTTTTATGTCT

SEQ ID NO: 23 - protein, 125 aa, artificial sequence
GTTTAAGAGCTATGCTGGAAACAGCATAGCAAGTTTAAATAAGGCTAGTCCGTTATCAACTTGAAAAAGTGGCACCGAGTCGGTGCCTGAATGCCTGCGAGCATCTTTTTTTGTTTTTTATGTCT

SEQ ID NO: 24 - protein, 173 aa, artificial sequence
GTTTAAGAGCTATGCTGGAAACAGCATAGCAAGTTTAAATAAGGCTAGTCCGTTATCAACTTGAAAAAGTGGCACCGAGTCGGTGCGGGAGCCTGAATGCCTGCGAGCATCGCCTGCTGCGCTGAATGCCTGCGAGCATCCGCAGCAGTTCCCTTTTTTTGTTTTTTATGTCT

SEQ ID NO: 25 - protein, 1367 aa, artificial sequence
DKKYSIGLAIGTNSVGWAVITDEYKVPSKKFKVLGNTDRHSIKKNLIGALLFDSGETAEATRLKRTARRRYTRRKNRICYLQEIFSNEMAKVDDSFFHRLEESFLVEEDKKHERHPIFGNIVDEVAYHEKYPTIYHLRKKLVDSTDKADLRLIYLALAHMIKFRGHFLIEGDLNPDNSDVDKLFIQLVQTYNQLFEENPINASGVDAKAILSARLSKSRRLENLIAQLPGEKKNGLFGNLIALSLGLTPNFKSNFDLAEDAKLQLSKDTYDDDLDNLLAQIGDQYADLFLAAKNLSDAILLSDILRVNTEITKAPLSASMIKRYDEHHQDLTLLKALVRQQLPEKYKEIFFDQSKNGYAGYIDGGASQEEFYKFIKPILEKMDGTEELLVKLNREDLLRKQRTFDNGSIPHQIHLGELHAILRRQEDFYPFLKDNREKIEKILTFRIPYYVGPLARGNSRFAWMTRKSEETITPWNFEEVVDKGASAQSFIERMTNFDKNLPNEKVLPKHSLLYEYFTVYNELTKVKYVTEGMRKPAFLSGEQKKAIVDLLFKTNRKVTVKQLKEDYFKKIECFDSVEISGVEDRFNASLGTYHDLLKIIKDKDFLDNEENEDILEDIVLTLTLFEDREMIEERLKTYAHLFDDKVMKQLKRRRYTGWGRLSRKLINGIRDKQSGKTILDFLKSDGFANRNFMQLIHDDSLTFKEDIQKAQVSGQGDSLHEHIANLAGSPAIKKGILQTVKVVDELVKVMGRHKPENIVIEMARENQTTQKGQKNSRERMKRIEEGIKELGSQILKEHPVENTQLQNEKLYLYYLQNGRDMYVDQELDINRLSDYDVDHIVPQSFLKDDSIDNKVLTRSDKNRGKSDNVPSEEVVKKMKNYWRQLLNAKLITQRKFDNLTKAERGGLSELDKAGFIKRQLVETRQITKHVAQILDSRMNTKYDENDKLIREVKVITLKSKLVSDFRKDFQFYKVREINNYHHAHDAYLNAVVGTALIKKYPKLESEFVYGDYKVYDVRKMIAKSEQEIGKATAKYFFYSNIMNFFKTEITLANGEIRKRPLIETNGETGEIVWDKGRDFATVRKVLSMPQVNIVKKTEVQTGGFSKESILPKRNSDKLIARKKDWDPKKYGGFDSPTVAYSVLVVAKVEKGKSKKLKSVKELLGITIMERSSFEKNPIDFLEAKGYKEVKKDLIIKLPKYSLFELENGRKRMLASAGELQKGNELALPSKYVNFLYLASHYEKLKGSPEDNEQKQLFVEQHKHYLDEIIEQISEFSKRVILADANLDKVLSAYNKHRDKPIREQAENIIHLFTLTNLGAPAAFKYFDTTIDRKRYTSTKEVLDATLIHQSITGLYETRIDLSQLGGD

SEQ ID NO: 26 - protein, 228 aa, artificial sequence
SSETGPVAVDPTLRRRIEPHEFEVFFDPRELRKETCLLYEINWGGRHSIWRHTSQNTNKHVEVNFIEKFTTERYFCPNTRCSITWFLSWSPCGECSRAITEFLSRYPHVTLFIYIARLYHHADPRNRQGLRDLISSGVTIQIMTEQESGYCWRNFVNYSPSNEAHWPRYPHLWVRLYVLELYCIILGLPPCLNILRRKQPQLTFFTIALQSCHYQRLPPHILWATGLK

SEQ ID NO: 27 - protein, 228 aa, artificial sequence
SSETGPVAVDPTLRRRIEPHEFEVFFDPRELRKETCLLYEINWGGRHSIWRHTSQNTNKHVEVNFIEKFTTERYFCPNTRCSITWFLSYSPCGECSRAITEFLSRYPHVTLFIYIARLYHHADPENRQGLRDLISSGVTIQIMTEQESGYCWRNFVNYSPSNEAHWPRYPHLWVRLYVLELYCIILGLPPCLNILRRKQPQLTFFTIALQSCHYQRLPPHILWATGLK

SEQ ID NO: 28 - protein, 228 aa, artificial sequence
SSETGPVAVDPTLRRRIEPHEFEVFFDPRELRKETCLLYEINWGGRHSIWRHTSQNTNKHVEVNFIEKFTTERYFCPNTRCSITWFLSYSPCGECSRAITEFLSRYPHVTLFIYIARLYHHADPRNRQGLEDLISSGVTIQIMTEQESGYCWRNFVNYSPSNEAHWPRYPHLWVRLYVLELYCIILGLPPCLNILRRKQPQLTFFTIALQSCHYQRLPPHILWATGLK

SEQ ID NO: 29 - protein, 228 aa, artificial sequence
SSETGPVAVDPTLRRRIEPHEFEVFFDPRELRKETCLLYEINWGGRHSIWRHTSQNTNKHVEVNFIEKFTTERYFCPNTRCSITWFLSWSPCGECSRAITEFLSRYPHVTLFIYIARLYHHADPENRQGLEDLISSGVTIQIMTEQESGYCWRNFVNYSPSNEAHWPRYPHLWVRLYVLELYCIILGLPPCLNILRRKQPQLTFFTIALQSCHYQRLPPHILWATGLK

SEQ ID NO: 30 - protein, 228 aa, artificial sequence
SSETGPVAVDPTLRRRIEPHEFEVFFDPRELRKETCLLYEINWGGRHSIWRHTSQNTNKHVEVNFIEKFTTERYFCPNTRCSITWFLSYSPCGECSRAITEFLSRYPHVTLFIYIARLYHHADPENRQGLEDLISSGVTIQIMTEQESGYCWRNFVNYSPSNEAHWPRYPHLWVRLYVLELYCIILGLPPCLNILRRKQPQLTFFTIALQSCHYQRLPPHILWATGLK

SEQ ID NO: 31 - protein, 83 aa, artificial sequence
TNLSDIIEKETGKQLVIQESILMLPEEVEEVIGNKPESDILVHTAYDESTDENVMLLTSDAPEYKPWALVIQDSNGENKIKML

SEQ ID NO: 32 - protein, 166 aa, artificial sequence
SEVEFSHEYWMRHALTLAKRAWDEREVPVGAVLVHNNRVIGEGWNRPIGRHDPTAHAEIMALRQGGLVMQNYRLIDATLYVTLEPCVMCAGAMIHSRIGRVVFGARDAKTGAAGSLMDVLHHPGMNHRVEITEGILADECAALLSDFFRMRRQEIKAQKKAQSSTD

SEQ ID NO: 33 - protein, 166 aa, artificial sequence
SEVEFSHEYWMRHALTLAKRARDEREVPVGAVLVLNNRVIGEGWNRAIGLHDPTAHAEIMALRQGGLVMQNYRLIDATLYVTFEPCVMCAGAMIHSRIGRVVFGVRNAKTGAAGSLMDVLHYPGMNHRVEITEGILADECAALLCYFFRMPRQVFNAQKKAQSSTD

SEQ ID NO: 34 - protein, 116 aa, artificial sequence
ASNFTQFVLVDNGGTGDVTVAPSNFANGIAEWISSNSRSQAYKVTCSVRQSSAQNRKYTIKVEVPKGAWRSYLNMELTIPIFATNSDCELIVKAMQGLLKDGNPIPSAIAANSGIY

SEQ ID NO: 35 - protein, 121 aa, artificial sequence
SKTIVLSVGEATRTLTEIQSTADRQIFEEKVGPLVGRLRLTASLRQNGAKTAYRVNLKLDQADVVDSGLPKVRYTQVWSHDVTIVANSTEASRKSLYDLTKSLVATSQVEDLVVNLVPLGR

SEQ ID NO: 36 - protein, 22 aa, artificial sequence
GNARTRRRERRAEKQAQWKAAN

SEQ ID NO: 37 - protein, 61 aa, artificial sequence
KSIRCKNCNKLLFKADSFDHIEIRCPRCKRHIIMLNACEHPTEKHCGKREKITHSDETVRY

SEQ ID NO: 38 - protein, 18 aa, artificial sequence
EGRGSLLTCGDVEENPGP

SEQ ID NO: 39 - protein, 16 aa, artificial sequence
KRPAATKKAGQAKKKK

SEQ ID NO: 40 - protein, 7 aa, artificial sequence
PKKKRKV

SEQ ID NO: 41 - protein, 16 aa, artificial sequence
SGSETPGTSESATPES

SEQ ID NO: 42 - protein, 32 aa, artificial sequence
SGGSSGGSSGSETPGTSESATPESSGGSSGGS

SEQ ID NO: 43 - protein, 32 aa, artificial sequence; identical to SEQ ID NO: 42

SEQ ID NO: 44 - protein, 469 aa, artificial sequence
GTTTAAGAGCTATGCTGGAAACAGCATAGCAAGTTTAAATAAGGCTAGTCCGTTATCAACTTGAAAAAGTGGCACCGAGTCGGTGCTTTTTTTGTTTTTTATGTCTGACCAAGCCCGTTATTCTGACAGTTCTGGTGCTCAACACATTTATATTTATCAAGGAGCACATTGTTACTCACTGCTAGGAGGGAATCGAACTAGGAATATTGATCAGAGGAACTACGAGAGAGCTGAAGATAACTGCCCTCTAGCTCTCACTGATCTGGGTCGCATAGTGAGATGCAGCCCACGTGAGTTCAGCAACGGTCTAGCGCTGGGCTTTTAGGCCCGCATGATCGGGCTTTTGTCGGGTGGTCGACGTGTTCACGATTGGGGAGAGCAACGCAGCAGTTCCTCTTAGTTTAGTCCCACCTCGCCTGTCCAGCAGAGTTCTGACCGGTTTATAAACTCGCTTGCTGCATCAGACTTG

SEQ ID NO: 45 - protein, 528 aa, artificial sequence
GTTTAAGAGCTATGCTGGAAACAGCATAGCAAGTTTAAATAAGGCTAGTCCGTTATCAACTTGAAAAAGTGGCACCGAGTCGGTGCGGGAGCGCCCTGAAGAAGGGCGCCTGCTGCGGCCCTGAAGAAGGGCCGCAGCAGTTCCCTTTTTTTGTTTTTTATGTCTGACCAAGCCCGTTATTCTGACAGTTCTGGTGCTCAACACATTTATATTTATCAAGGAGCACATTGTTACTCACTGCTAGGAGGGAATCGAACTAGGAATATTGATCAGAGGAACTACGAGAGAGCTGAAGATAACTGCCCTCTAGCTCTCACTGATCTGGGTCGCATAGTGAGATGCAGCCCACGTGAGTTCAGCAACGGTCTAGCGCTGGGCTTTTAGGCCCGCATGATCGGGCTTTTGTCGGGTGGTCGACGTGTTCACGATTGGGGAGAGCAACGCAGCAGTTCCTCTTAGTTTAGTCCCACCTCGCCTGTCCAGCAGAGTTCTGACCGGTTTATAAACTCGCTTGCTGCATCAGACTTG

SEQ ID NO: 46 - protein, 7095 aa, artificial sequence
ATGGACAAGAAGTACTCGATCGGCCTCGCCATTGGGACTAACTCTGTTGGCTGGGCCGTGATCACCGACGAGTACAAGGTGCCCTCAAAGAAGTTCAAGGTCCTGGGCAACACCGATCGGCATTCCATCAAGAAGAATCTCATTGGCGCTCTCCTGTTCGACAGCGGCGAGACGGCTGAGGCTACGCGGCTCAAGCGCACCGCCCGCAGGCGGTACACGCGCAGGAAGAATCGCATCTGCTACCTGCAGGAGATTTTCTCCAACGAGATGGCGAAGGTTGACGATTCTTTCTTCCACAGGCTGGAGGAGTCATTCCTCGTGGAGGAGGATAAGAAGCACGAGCGGCATCCAATCTTCGGCAACATTGTCGACGAGGTTGCCTACCACGAGAAGTACCCTACGATCTACCATCTGCGGAAGAAGCTCGTGGACTCCACAGATAAGGCGGACCTCCGCCTGATCTACCTCGCTCTGGCCCACATGATTAAGTTCAGGGGCCATTTCCTGATCGAGGGGGATCTCAACCCGGACAATAGCGATGTTGACAAGCTGTTCATCCAGCTCGTGCAGACGTACAACCAGCTCTTCGAGGAGAACCCCATTAATGCGTCAGGCGTCGACGCGAAGGCTATCCTGTCCGCTAGGCTCTCGAAGTCTCGGCGCCTCGAGAACCTGATCGCCCAGCTGCCGGGCGAGAAGAAGAACGGCCTGTTCGGGAATCTCATTGCGCTCAGCCTGGGGCTCACGCCCAACTTCAAGTCGAATTTCGATCTCGCTGAGGACGCCAAGCTGCAGCTCTCCAAGGACACATACGACGATGACCTGGATAACCTCCTGGCCCAGATCGGCGATCAGTACGCGGACCTGTTCCTCGCTGCCAAGAATCTGTCGGACGCCATCCTCCTGTCTGATATTCTCAGGGTGAACACCGAGATTACGAAGGCTCCGCTCTCAGCCTCCATGATCAAGCGCTACGACGAGCACCATCAGGATCTGACCCTCCTGAAGGCGCTGGTCAGGCAGCAGCTCCCCGAGAAGTACAAGGAGATCTTCTTCGATCAGTCGAAGAACGGCTACGCTGGGTACATTGACGGCGGGGCCTCTCAGGAGGAGTTCTACAAGTTCATCAAGCCGATTCTGGAGAAGATGGACGGCACGGAGGAGCTGCTGGTGAAGCTCAATCGCGAGGACCTCCTGAGGAAGCAGCGGACATTCGATAACGGCAGCATCCCACACCAGATTCATCTCGGGGAGCTGCACGCTATCCTGAGGAGGCAGGAGGACTTCTACCCTTTCCTCAAGGATAACCGCGAGAAGATCGAGAAGATTCTGACTTTCAGGATCCCGTACTACGTCGGCCCACTCGCTAGGGGCAACTCCCGCTTCGCTTGGATGACCCGCAAGTCAGAGGAGACGATCACGCCGTGGAACTTCGAGGAGGTGGTCGACAAGGGCGCTAGCGCTCAGTCGTTCATCGAGAGGATGACGAATTTCGACAAGAACCTGCCAAATGAGAAGGTGCTCCCTAAGCACTCGCTCCTGTACGAGTACTTCACAGTCTACAACGAGCTGACTAAGGTGAAGTATGTGACCGAGGGCATGAGGAAGCCGGCTTTCCTGTCTGGGGAGCAGAAGAAGGCCATCGTGGACCTCCTGTTCAAGACCAACCGGAAGGTCACGGTTAAGCAGCTCAAGGAGGACTACTTCAAGAAGATTGAGTGCTTCGATTCGGTCGAGATCTCTGGCGTTGAGGACCGCTTCAACGCCTCCCTGGGGACCTACCACGATCTCCTGAAGATCATTAAGGATAAGGACTTCCTGGACAACGAGGAGAATGAGGATATCCTCGAGGACATTGTGCTGACACTCACTCTGTTCGAGGACCGGGAGATGATCGAGGAGCGCCTGAAGACTTACGCCCATCTCTTCGATGACAAGGTCATGAAGCAGCTCAAGAGGAGGAGGTACACCGGCTGGGGGAGGCTGAGCAGGAAGCTCATCAACGGCATTCGGGACAAGCAGTCCGGGAAGACGATCCTCGACTTCCTGAAGAGCGATGGCTTCGCGAACCGCAATTTCATGCAGCTGATTCACGATGACAGCCTCACATTCAAGGAGGATATCCAGAAGGCTCAGGTGAGCGGCCAGGGGGACTCGCTGCACGAGCATATCGCGAACCTCGCTGGCTCGCCAGCTATCAAGAAGGGGATTCTGCAGACCGTGAAGGTTGTGGACGAGCTGGTGAAGGTCATGGGCAGGCACAAGCCTGAGAACATCGTCATTGAGATGGCCCGGGAGAATCAGACCACGCAGAAGGGCCAGAAGAACTCACGCGAGAGGATGAAGAGGATCGAGGAGGGCATTAAGGAGCTGGGGTCCCAGATCCTCAAGGAGCACCCGGTGGAGAACACGCAGCTGCAGAATGAGAAGCTCTACCTGTACTACCTCCAGAATGGCCGCGATATGTATGTGGACCAGGAGCTGGATATTAACAGGCTCAGCGATTACGACGTCGATCATATCGTTCCACAGTCATTCCTGAAGGATGACTCCATTGACAACAAGGTCCTCACCAGGTCGGACAAGAACCGGGGCAAGTCTGATAATGTTCCTTCAGAGGAGGTCGTTAAGAAGATGAAGAACTACTGGCGCCAGCTCCTGAATGCCAAGCTGATCACGCAGCGGAAGTTCGATAACCTCACAAAGGCTGAGAGGGGCGGGCTCTCTGAGCTGGACAAGGCGGGCTTCATCAAGAGGCAGCTGGTCGAGACACGGCAGATCACTAAGCACGTTGCGCAGATTCTCGACTCACGGATGAACACTAAGTACGATGAGAATGACAAGCTGATCCGCGAGGTGAAGGTCATCACCCTGAAGTCAAAGCTCGTCTCCGACTTCAGGAAGGATTTCCAGTTCTACAAGGTTCGGGAGATCAACAATTACCACCATGCCCATGACGCGTACCTGAACGCGGTGGTCGGCACAGCTCTGATCAAGAAGTACCCAAAGCTCGAGAGCGAGTTCGTGTACGGGGACTACAAGGTTTACGATGTGAGGAAGATGATCGCCAAGTCGGAGCAGGAGATTGGCAAGGCTACCGCCAAGTACTTCTTCTACTCTAACATTATGAATTTCTTCAAGACAGAGATCACTCTGGCCAATGGCGAGATCCGGAAGCGCCCCCTCATCGAGACGAACGGCGAGACGGGGGAGATCGTGTGGGACAAGGGCAGGGATTTCGCGACCGTCAGGAAGGTTCTCTCCATGCCACAAGTGAATATCGTCAAGAAGACAGAGGTCCAGACTGGCGGGTTCTCTAAGGAGTCAATTCTGCCTAAGCGGAACAGCGACAAGCTCATCGCCCGCAAGAAGGACTGGGATCCGAAGAAGTACGGCGGGTTCGACAGCCCCACTGTGGCCTACTCGGTCCTGGTTGTGGCGAAGGTTGAGAAGGGCAAGTCCAAGAAGCTCAAGAGCGTGAAGGAGCTGCTGGGGATCACGATTATGGAGCGCTCCAGCTTCGAGAAGAACCCGATCGATTTCCTGGAGGCGAAGGGCTACAAGGAGGTGAAGAAGGACCTGATCATTAAGCTCCCCAAGTACTCACTCTTCGAGCTGGAGAACGGCAGGAAGCGGATGCTGGCTTCCGCTGGCGAGCTGCAGAAGGGGAACGAGCTGGCTCTGCCGTCCAAGTATGTGAACTTCCTCTACCTGGCCTCCCACTACGAGAAGCTCAAGGGCAGCCCCGAGGACAACGAGCAGAAGCAGCTGTTCGTCGAGCAGCACAAGCATTACCTCGACGAGATCATTGAGCAGATTTCCGAGTTCTCCAAGCGCGTGATCCTGGCCGACGCGAATCTGGATAAGGTCCTCTCCGCGTACAACAAGCACCGCGACAAGCCAATCAGGGAGCAGGCTGAGAATATCATTCATCTCTTCACCCTGACGAACCTCGGCGCCCCTGCTGCTTTCAAGTACTTCGACACAACTATCGATCGCAAGAGGTACACAAGCACTAAGGAGGTCCTGGACGCGACCCTCATCCACCAGTCGATTACCGGCCTCTACGAGACGCGCATCGACCTGTCTCAGCTCGGGGGCGACTCCGGCGGCAGCCCAAAGAAGAAGCGGAAGGTGTCTGGAGGTTCTCCTAAGAAAAAGAGAAAAGTGTCCGGCGGCTCCCCGAAGAAGAAGCGCAAGGTGGAATTCGAGGGCAGAGGAAGTCTTCTAACATGCGGTGACGTGGAGGAGAATCCCGGCCCTGCCTCAAACTTCACCCAGTTCGTGCTCGTCGACAATGGCGGAACCGGCGATGTGACAGTCGCACCTTCCAACTTCGCCAATGGCATCGCGGAGTGGATTTCCAGCAACTCCAGGTCCCAGGCGTACAAGGTGACCTGCTCCGTCAGGCAGTCATCTGCGCAGAATCGCAAGTACACAATCAAGGTGGAGGTCCCTAAGGGCGCCTGGAGGTCCTACCTCAACATGGAGCTGACCATCCCGATTTTCGCCACAAATAGCGACTGCGAGCTGATCGTGAAGGCGATGCAGGGCCTCCTGAAGGATGGCAACCCGATCCCATCAGCGATTGCCGCGAATTCTGGCATCTACTCCGGCAGCGAGACGCCAGGCACCTCCGAGAGCGCTACGCCTGAATCCCCAAAGAAGAAGAGGAAGGTTTCATCGGAAACCGGCCCTGTTGCTGTTGACCCCACCCTGCGGCGGAGAATCGAGCCACACGAGTTCGAGGTGTTCTTCGACCCAAGGGAGCTCCGCAAGGAGACGTGCCTCCTGTACGAGATCAACTGGGGCGGCAGGCACTCCATCTGGAGGCACACCAGCCAAAACACCAACAAGCACGTGGAGGTCAACTTCATCGAGAAGTTCACCACCGAGAGGTACTTCTGCCCAAACACCCGCTGCTCCATCACCTGGTTCCTGTCCTGGAGCCCATGCGGCGAGTGCTCCAGGGCCATCACCGAGTTCCTCAGCCGCTACCCACACGTCACCCTGTTCATCTACATCGCCAGGCTCTACCACCACGCCGACCCAAGGAACAGGCAGGGCCTCCGCGACCTGATCTCCAGCGGCGTGACCATCCAAATCATGACCGAGCAGGAGTCCGGCTACTGCTGGAGGAACTTCGTCAACTACTCCCCAAGCAACGAGGCCCACTGGCCAAGGTACCCACACCTCTGGGTGCGCCTCTACGTGCTCGAGCTGTACTGCATCATCCTCGGCCTGCCACCATGCCTCAACATCCTGAGGCGCAAGCAACCACAGCTGACCTTCTTCACCATCGCCCTCCAAAGCTGCCACTACCAGAGGCTCCCACCACACATCCTGTGGGCTACCGGCCTCAAGTCGGGGGGGAGCACCAACCTGTCCGACATCATCGAGAAGGAGACGGGCAAGCAACTCGTGATCCAGGAGAGCATCCTCATGCTGCCAGAGGAGGTGGAGGAGGTCATCGGCAACAAGCCAGAGTCCGACATCCTGGTGCACACCGCCTACGACGAGTCCACCGACGAGAACGTCATGCTCCTGACCAGCGACGCCCCAGAGTACAAGCCATGGGCCCTCGTCATCCAGGACAGCAACGGGGAGAACAAGATCAAGATGCTGTCGGGGGGGAGCAAGCGGCCAGCGGCGACGAAGAAGGCGGGGCAGGCGAAGAAGAAGAAGGAGGGCAGAGGAAGTCTTCTAACATGCGGTGACGTGGAGGAGAATCCCGGCCCTTCCGAGGTGGAGTTCTCTCACGAGTATTGGATGAGGCACGCTCTTACACTTGCTAAGAGAGCTTGGGACGAAAGAGAAGTGCCAGTTGGCGCCGTTCTTGTGCATAATAATAGGGTGATCGGCGAGGGTTGGAATAGACCAATTGGAAGGCATGATCCAACAGCTCACGCAGAGATTATGGCTCTCAGACAAGGCGGCCTCGTTATGCAGAACTACAGGCTCATTGACGCTACACTCTACGTGACACTCGAACCTTGCGTTATGTGCGCCGGAGCTATGATTCATTCTAGGATTGGCAGGGTCGTGTTTGGAGCTAGGGACGCTAAAACAGGAGCCGCCGGATCTCTTATGGACGTGTTGCATCATCCAGGCATGAACCATAGGGTGGAGATTACAGAGGGCATTCTTGCAGACGAGTGCGCTGCTCTTCTTTCCGATTTCTTCAGGATGAGAAGGCAGGAGATTAAGGCCCAGAAGAAGGCTCAGTCTTCTACAGATAGCGGAGGATCTTCCGGAGGATCTAGCGGCTCCGAGACACCAGGAACATCCGAAAGCGCTACACCAGAATCTAGCGGAGGCTCTTCCGGAGGATCTTCTGAAGTGGAGTTCTCCCACGAGTATTGGATGAGGCACGCTCTTACACTTGCTAAAAGGGCTAGGGACGAAAGGGAAGTTCCAGTTGGAGCTGTTCTCGTGCTCAATAACAGGGTGATTGGCGAGGGTTGGAATAGAGCCATTGGACTCCATGATCCAACAGCTCACGCAGAGATTATGGCTCTTAGACAAGGCGGCCTCGTTATGCAGAATTACAGACTCATCGACGCCACACTCTACGTTACCTTCGAACCTTGCGTTATGTGCGCCGGAGCTATGATCCATTCTAGGATTGGCAGGGTCGTGTTCGGCGTTAGAAACGCTAAGACAGGAGCTGCAGGCTCTCTTATGGACGTTCTTCATTACCCAGGCATGAATCATAGAGTGGAGATCACAGAAGGCATTCTTGCAGACGAGTGCGCAGCTCTCCTTTGCTATTTCTTCAGGATGCCGAGGCAAGTTTTCAACGCTCAGAAGAAGGCCCAGTCTTCTACAGATTCCGGCGGATCTTCCGGAGGATCTAGCGGCTCCGAGACACCAGGAACATCCGAATCCGCTACACCAGAGTCTTCTGGAGGATCTAGCGGAGGATCTGGCAACGCCAGGACCAGGAGGAGGGAGAGGAGGGCCGAGAAGCAGGCCCAGTGGAAGGCCGCCAACTCCGGCGGCAGCCCAAAGAAGAAGCGGAAGGTGTCTGGAGGTTCTCCTAAGAAAAAGAGAAAAGTGTCCGGCGGCTCCCCGAAGAAGAAGCGCAAGGTGTAG

SEQ ID NO: 47 - protein, 7095 aa, artificial sequence
ATGGACAAGAAGTACTCGATCGGCCTCGCCATTGGGACTAACTCTGTTGGCTGGGCCGTGATCACCGACGAGTACAAGGTGCCCTCAAAGAAGTTCAAGGTCCTGGGCAACACCGATCGGCATTCCATCAAGAAGAATCTCATTGGCGCTCTCCTGTTCGACAGCGGCGAGACGGCTGAGGCTACGCGGCTCAAGCGCACCGCCCGCAGGCGGTACACGCGCAGGAAGAATCGCATCTGCTACCTGCAGGAGATTTTCTCCAACGAGATGGCGAAGGTTGACGATTCTTTCTTCCACAGGCTGGAGGAGTCATTCCTCGTGGAGGAGGATAAGAAGCACGAGCGGCATCCAATCTTCGGCAACATTGTCGACGAGGTTGCCTACCACGAGAAGTACCCTACGATCTACCATCTGCGGAAGAAGCTCGTGGACTCCACAGATAAGGCGGACCTCCGCCTGATCTACCTCGCTCTGGCCCACATGATTAAGTTCAGGGGCCATTTCCTGATCGAGGGGGATCTCAACCCGGACAATAGCGATGTTGACAAGCTGTTCATCCAGCTCGTGCAGACGTACAACCAGCTCTTCGAGGAGAACCCCATTAATGCGTCAGGCGTCGACGCGAAGGCTATCCTGTCCGCTAGGCTCTCGAAGTCTCGGCGCCTCGAGAACCTGATCGCCCAGCTGCCGGGCGAGAAGAAGAACGGCCTGTTCGGGAATCTCATTGCGCTCAGCCTGGGGCTCACGCCCAACTTCAAGTCGAATTTCGATCTCGCTGAGGACGCCAAGCTGCAGCTCTCCAAGGACACATACGACGATGACCTGGATAACCTCCTGGCCCAGATCGGCGATCAGTACGCGGACCTGTTCCTCGCTGCCAAGAATCTGTCGGACGCCATCCTCCTGTCTGATATTCTCAGGGTGAACACCGAGATTACGAAGGCTCCGCTCTCAGCCTCCATGATCAAGCGCTACGACGAGCACCATCAGGATCTGACCCTCCTGAAGGCGCTGGTCAGGCAGCAGCTCCCCGAGAAGTACAAGGAGATCTTCTTCGATCAGTCGAAGAACGGCTACGCTGGGTACATTGACGGCGGGGCCTCTCAGGAGGAGTTCTACAAGTTCATCAAGCCGATTCTGGAGAAGATGGACGGCACGGAGGAGCTGCTGGTGAAGCTCAATCGCGAGGACCTCCTGAGGAAGCAGCGGACATTCGATAACGGCAGCATCCCACACCAGATTCATCTCGGGGAGCTGCACGCTATCCTGAGGAGGCAGGAGGACTTCTACCCTTTCCTCAAGGATAACCGCGAGAAGATCGAGAAGATTCTGACTTTCAGGATCCCGTACTACGTCGGCCCACTCGCTAGGGGCAACTCCCGCTTCGCTTGGATGACCCGCAAGTCAGAGGAGACGATCACGCCGTGGAACTTCGAGGAGGTGGTCGACAAGGGCGCTAGCGCTCAGTCGTTCATCGAGAGGATGACGAATTTCGACAAGAACCTGCCAAATGAGAAGGTGCTCCCTAAGCACTCGCTCCTGTACGAGTACTTCACAGTCTACAACGAGCTGACTAAGGTGAAGTATGTGACCGAGGGCATGAGGAAGCCGGCTTTCCTGTCTGGGGAGCAGAAGAAGGCCATCGTGGACCTCCTGTTCAAGACCAACCGGAAGGTCACGGTTAAGCAGCTCAAGGAGGACTACTTCAAGAAGATTGAGTGCTTCGATTCGGTCGAGATCTCTGGCGTTGAGGACCGCTTCAACGCCTCCCTGGGGACCTACCACGATCTCCTGAAGATCATTAAGGATAAGGACTTCCTGGACAACGAGGAGAATGAGGATATCCTCGAGGACATTGTGCTGACACTCACTCTGTTCGAGGACCGGGAGATGATCGAGGAGCGCCTGAAGACTTACGCCCATCTCTTCGATGACAAGGTCATGAAGCAGCTCAAGAGGAGGAGGTACACCGGCTGGGGGAGGCTGAGCAGGAAGCTCATCAACGGCATTCGGGACAAGCAGTCCGGGAAGACGATCCTCGACTTCCTGAAGAGCGATGGCTTCGCGAACCGCAATTTCATGCAGCTGATTCACGATGACAGCCTCACATTCAAGGAGGATATCCAGAAGGCTCAGGTGAGCGGCCAGGGGGACTCGCTGCACGAGCATATCGCGAACCTCGCTGGCTCGCCAGCTATCAAGAAGGGGATTCTGCAGACCGTGAAGGTTGTGGACGAGCTGGTGAAGGTCATGGGCAGGCACAAGCCTGAGAACATCGTCATTGAGATGGCCCGGGAGAATCAGACCACGCAGAAGGGCCAGAAGAACTCACGCGAGAGGATGAAGAGGATCGAGGAGGGCATTAAGGAGCTGGGGTCCCAGATCCTCAAGGAGCACCCGGTGGAGAACACGCAGCTGCAGAATGAGAAGCTCTACCTGTACTACCTCCAGAATGGCCGCGATATGTATGTGGACCAGGAGCTGGATATTAACAGGCTCAGCGATTACGACGTCGATCATATCGTTCCACAGTCATTCCTGAAGGATGACTCCATTGACAACAAGGTCCTCACCAGGTCGGACAAGAACCGGGGCAAGTCTGATAATGTTCCTTCAGAGGAGGTCGTTAAGAAGATGAAGAACTACTGGCGCCAGCTCCTGAATGCCAAGCTGATCACGCAGCGGAAGTTCGATAACCTCACAAAGGCTGAGAGGGGCGGGCTCTCTGAGCTGGACAAGGCGGGCTTCATCAAGAGGCAGCTGGTCGAGACACGGCAGATCACTAAGCACGTTGCGCAGATTCTCGACTCACGGATGAACACTAAGTACGATGAGAATGACAAGCTGATCCGCGAGGTGAAGGTCATCACCCTGAAGTCAAAGCTCGTCTCCGACTTCAGGAAGGATTTCCAGTTCTACAAGGTTCGGGAGATCAACAATTACCACCATGCCCATGACGCGTACCTGAACGCGGTGGTCGGCACAGCTCTGATCAAGAAGTACCCAAAGCTCGAGAGCGAGTTCGTGTACGGGGACTACAAGGTTTACGATGTGAGGAAGATGATCGCCAAGTCGGAGCAGGAGATTGGCAAGGCTACCGCCAAGTACTTCTTCTACTCTAACATTATGAATTTCTTCAAGACAGAGATCACTCTGGCCAATGGCGAGATCCGGAAGCGCCCCCTCATCGAGACGAACGGCGAGACGGGGGAGATCGTGTGGGACAAGGGCAGGGATTTCGCGACCGTCAGGAAGGTTCTCTCCATGCCACAAGTGAATATCGTCAAGAAGACAGAGGTCCAGACTGGCGGGTTCTCTAAGGAGTCAATTCGGCCTAAGCGGAACAGCGACAAGCTCATCGCCCGCAAGAAGGACTGGGATCCGAAGAAGTACGGCGGGTTCGTCAGCCCCACTGTGGCCTACTCGGTCCTGGTTGTGGCGAAGGTTGAGAAGGGCAAGTCCAAGAAGCTCAAGAGCGTGAAGGAGCTGCTGGGGATCACGATTATGGAGCGCTCCAGCTTCGAGAAGAACCCGATCGATTTCCTGGAGGCGAAGGGCTACAAGGAGGTGAAGAAGGACCTGATCATTAAGCTCCCCAAGTACTCACTCTTCGAGCTGGAGAACGGCAGGAAGCGGATGCTGGCTTCCGCTCGCTTCCTGCAGAAGGGGAACGAGCTGGCTCTGCCGTCCAAGTATGTGAACTTCCTCTACCTGGCCTCCCACTACGAGAAGCTCAAGGGCAGCCCCGAGGACAACGAGCAGAAGCAGCTGTTCGTCGAGCAGCACAAGCATTACCTCGACGAGATCATTGAGCAGATTTCCGAGTTCTCCAAGCGCGTGATCCTGGCCGACGCGAATCTGGATAAGGTCCTCTCCGCGTACAACAAGCACCGCGACAAGCCAATCAGGGAGCAGGCTGAGAATATCATTCATCTCTTCACCCTGACGAACCTCGGCGCCCCTCGTGCTTTCAAGTACTTCGACACAACTATCGATCGCAAGGTATACAGAAGCACTAAGGAGGTCCTGGACGCGACCCTCATCCACCAGTCGATTACCGGCCTCTACGAGACGCGCATCGACCTGTCTCAGCTCGGGGGCGACTCCGGCGGCAGCCCAAAGAAGAAGCGGAAGGTGTCTGGAGGTTCTCCTAAGAAAAAGAGAAAAGTGTCCGGCGGCTCCCCGAAGAAGAAGCGCAAGGTGGAATTCGAGGGCAGAGGAAGTCTTCTAACATGCGGTGACGTGGAGGAGAATCCCGGCCCTGCCTCAAACTTCACCCAGTTCGTGCTCGTCGACAATGGCGGAACCGGCGATGTGACAGTCGCACCTTCCAACTTCGCCAATGGCATCGCGGAGTGGATTTCCAGCAACTCCAGGTCCCAGGCGTACAAGGTGACCTGCTCCGTCAGGCAGTCATCTGCGCAGAATCGCAAGTACACAATCAAGGTGGAGGTCCCTAAGGGCGCCTGGAGGTCCTACCTCAACATGGAGCTGACCATCCCGATTTTCGCCACAAATAGCGACTGCGAGCTGATCGTGAAGGCGATGCAGGGCCTCCTGAAGGATGGCAACCCGATCCCATCAGCGATTGCCGCGAATTCTGGCATCTACTCCGGCAGCGAGACGCCAGGCACCTCCGAGAGCGCTACGCCTGAATCCCCAAAGAAGAAGAGGAAGGTTTCATCGGAAACCGGCCCTGTTGCTGTTGACCCCACCCTGCGGCGGAGAATCGAGCCACACGAGTTCGAGGTGTTCTTCGACCCAAGGGAGCTCCGCAAGGAGACGTGCCTCCTGTACGAGATCAACTGGGGCGGCAGGCACTCCATCTGGAGGCACACCAGCCAAAACACCAACAAGCACGTGGAGGTCAACTTCATCGAGAAGTTCACCACCGAGAGGTACTTCTGCCCAAACACCCGCTGCTCCATCACCTGGTTCCTGTCCTGGAGCCCATGCGGCGAGTGCTCCAGGGCCATCACCGAGTTCCTCAGCCGCTACCCACACGTCACCCTGTTCATCTACATCGCCAGGCTCTACCACCACGCCGACCCAAGGAACAGGCAGGGCCTCCGCGACCTGATCTCCAGCGGCGTGACCATCCAAATCATGACCGAGCAGGAGTCCGGCTACTGCTGGAGGAACTTCGTCAACTACTCCCCAAGCAACGAGGCCCACTGGCCAAGGTACCCACACCTCTGGGTGCGCCTCTACGTGCTCGAGCTGTACTGCATCATCCTCGGCCTGCCACCATGCCTCAACATCCTGAGGCGCAAGCAACCACAGCTGACCTTCTTCACCATCGCCCTCCAAAGCTGCCACTACCAGAGGCTCCCACCACACATCCTGTGGGCTACCGGCCTCAAGTCGGGGGGGAGCACCAACCTGTCCGACATCATCGAGAAGGAGACGGGCAAGCAACTCGTGATCCAGGAGAGCATCCTCATGCTGCCAGAGGAGGTGGAGGAGGTCATCGGCAACAAGCCAGAGTCCGACATCCTGGTGCACACCGCCTACGACGAGTCCACCGACGAGAACGTCATGCTCCTGACCAGCGACGCCCCAGAGTACAAGCCATGGGCCCTCGTCATCCAGGACAGCAACGGGGAGAACAAGATCAAGATGCTGTCGGGGGGGAGCAAGCGGCCAGCGGCGACGAAGAAGGCGGGGCAGGCGAAGAAGAAGAAGGAGGGCAGAGGAAGTCTTCTAACATGCGGTGACGTGGAGGAGAATCCCGGCCCTTCCGAGGTGGAGTTCTCTCACGAGTATTGGATGAGGCACGCTCTTACACTTGCTAAGAGAGCTTGGGACGAAAGAGAAGTGCCAGTTGGCGCCGTTCTTGTGCATAATAATAGGGTGATCGGCGAGGGTTGGAATAGACCAATTGGAAGGCATGATCCAACAGCTCACGCAGAGATTATGGCTCTCAGACAAGGCGGCCTCGTTATGCAGAACTACAGGCTCATTGACGCTACACTCTACGTGACACTCGAACCTTGCGTTATGTGCGCCGGAGCTATGATTCATTCTAGGATTGGCAGGGTCGTGTTTGGAGCTAGGGACGCTAAAACAGGAGCCGCCGGATCTCTTATGGACGTGTTGCATCATCCAGGCATGAACCATAGGGTGGAGATTACAGAGGGCATTCTTGCAGACGAGTGCGCTGCTCTTCTTTCCGATTTCTTCAGGATGAGAAGGCAGGAGATTAAGGCCCAGAAGAAGGCTCAGTCTTCTACAGATAGCGGAGGATCTTCCGGAGGATCTAGCGGCTCCGAGACACCAGGAACATCCGAAAGCGCTACACCAGAATCTAGCGGAGGCTCTTCCGGAGGATCTTCTGAAGTGGAGTTCTCCCACGAGTATTGGATGAGGCACGCTCTTACACTTGCTAAAAGGGCTAGGGACGAAAGGGAAGTTCCAGTTGGAGCTGTTCTCGTGCTCAATAACAGGGTGATTGGCGAGGGTTGGAATAGAGCCATTGGACTCCATGATCCAACAGCTCACGCAGAGATTATGGCTCTTAGACAAGGCGGCCTCGTTATGCAGAATTACAGACTCATCGACGCCACACTCTACGTTACCTTCGAACCTTGCGTTATGTGCGCCGGAGCTATGATCCATTCTAGGATTGGCAGGGTCGTGTTCGGCGTTAGAAACGCTAAGACAGGAGCTGCAGGCTCTCTTATGGACGTTCTTCATTACCCAGGCATGAATCATAGAGTGGAGATCACAGAAGGCATTCTTGCAGACGAGTGCGCAGCTCTCCTTTGCTATTTCTTCAGGATGCCGAGGCAAGTTTTCAACGCTCAGAAGAAGGCCCAGTCTTCTACAGATTCCGGCGGATCTTCCGGAGGATCTAGCGGCTCCGAGACACCAGGAACATCCGAATCCGCTACACCAGAGTCTTCTGGAGGATCTAGCGGAGGATCTGGCAACGCCAGGACCAGGAGGAGGGAGAGGAGGGCCGAGAAGCAGGCCCAGTGGAAGGCCGCCAACTCCGGCGGCAGCCCAAAGAAGAAGCGGAAGGTGTCTGGAGGTTCTCCTAAGAAAAAGAGAAAAGTGTCCGGCGGCTCCCCGAAGAAGAAGCGCAAGGTGTAG

SEQ ID NO: 48 - protein, 1368 aa, artificial sequence
MDKKYSIGLAIGTNSVGWAVITDEYKVPSKKFKVLGNTDRHSIKKNLIGALLFDSGETAEATRLKRTARRRYTRRKNRICYLQEIFSNEMAKVDDSFFHRLEESFLVEEDKKHERHPIFGNIVDEVAYHEKYPTIYHLRKKLVDSTDKADLRLIYLALAHMIKFRGHFLIEGDLNPDNSDVDKLFIQLVQTYNQLFEENPINASGVDAKAILSARLSKSRRLENLIAQLPGEKKNGLFGNLIALSLGLTPNFKSNFDLAEDAKLQLSKDTYDDDLDNLLAQIGDQYADLFLAAKNLSDAILLSDILRVNTEITKAPLSASMIKRYDEHHQDLTLLKALVRQQLPEKYKEIFFDQSKNGYAGYIDGGASQEEFYKFIKPILEKMDGTEELLVKLNREDLLRKQRTFDNGSIPHQIHLGELHAILRRQEDFYPFLKDNREKIEKILTFRIPYYVGPLARGNSRFAWMTRKSEETITPWNFEEVVDKGASAQSFIERMTNFDKNLPNEKVLPKHSLLYEYFTVYNELTKVKYVTEGMRKPAFLSGEQKKAIVDLLFKTNRKVTVKQLKEDYFKKIECFDSVEISGVEDRFNASLGTYHDLLKIIKDKDFLDNEENEDILEDIVLTLTLFEDREMIEERLKTYAHLFDDKVMKQLKRRRYTGWGRLSRKLINGIRDKQSGKTILDFLKSDGFANRNFMQLIHDDSLTFKEDIQKAQVSGQGDSLHEHIANLAGSPAIKKGILQTVKVVDELVKVMGRHKPENIVIEMARENQTTQKGQKNSRERMKRIEEGIKELGSQILKEHPVENTQLQNEKLYLYYLQNGRDMYVDQELDINRLSDYDVDHIVPQSFLKDDSIDNKVLTRSDKNRGKSDNVPSEEVVKKMKNYWRQLLNAKLITQRKFDNLTKAERGGLSELDKAGFIKRQLVETRQITKHVAQILDSRMNTKYDENDKLIREVKVITLKSKLVSDFRKDFQFYKVREINNYHHAHDAYLNAVVGTALIKKYPKLESEFVYGDYKVYDVRKMIAKSEQEIGKATAKYFFYSNIMNFFKTEITLANGEIRKRPLIETNGETGEIVWDKGRDFATVRKVLSMPQVNIVKKTEVQTGGFSKESIRPKRNSDKLIARKKDWDPKKYGGFVSPTVAYSVLVVAKVEKGKSKKLKSVKELLGITIMERSSFEKNPIDFLEAKGYKEVKKDLIIKLPKYSLFELENGRKRMLASARFLQKGNELALPSKYVNFLYLASHYEKLKGSPEDNEQKQLFVEQHKHYLDEIIEQISEFSKRVILADANLDKVLSAYNKHRDKPIREQAENIIHLFTLTNLGAPRAFKYFDTTIDRKVYRSTKEVLDATLIHQSITGLYETRIDLSQLGGD